European Patent Specification EP 3 512 537 B1, published November 1, 2023. Title: T-CELL IMMUNOTHERAPY. Applicant: Yu, Di Essand, Magnus Jin, Chuan Ramachandran, Mohanraj Ma, Jing. The sequence listing filed with the application follows.

SEQUENCE LISTING (16 sequences)

SEQ ID NO: 1 - protein, 144 aa, Helicobacter pylori
MKTFEILKHLQADAIVLFMKVHNFHWNVKGTDFFNVHKATEEIYEEFADMFDDLAERIVQLGHHPLVTLSEAIKLTRVKEETKTSFHSKDIFKEILEDYKYLEKEFKELSNTAEKEGDKVTVTYADDQLAKLQKSIWMLQAHLA

SEQ ID NO: 2 - protein, 144 aa, Helicobacter pylori
MKTFEILKHLQADAIVLFMKVHNFHWNVKGTDFFNVHKATEEIYEEFADMFDDLAERIVQLGHHPLVTLSEAIKLTRVKEETKTSFHSKDIFKEILEDYKHLEKEFKELSNTAEKEGDKVTVTYADDQLAKLQKSIWMLQAHLA

SEQ ID NO: 3 - protein, 144 aa, Helicobacter pylori
MKTFEILKHLQADAIVLFMKVHNFHWNVKGTDFFNVHKATEEIYEEFADMFDDLAERIVQLGHHPLVTLSEALKLTRVKEETKTSFHSKDIFKEILEDYKYLEKEFKELSNTAEKEGDKVTVTYADDQLAKLQKSIWMLQAHLA

SEQ ID NO: 4 - protein, 144 aa, Helicobacter pylori
MKTFEILKHLQADAIVLFMKVHNFHWNVKGTDFFNVHKATEEIYEEFADMFDDLAERIVQLGHHPLVTLSEALKLTRVKEETKTSFHSKDIFKEILEDYKHLEKEFKELSNTAEKEGDKVTVTYADDQLAKLQKSIWMLQAHLA

SEQ ID NO: 5 - protein, 144 aa, Helicobacter pylori
MKTFEILKHLQADAIVLFMKVHNFHWNVKGTDFFNVHKATEEIYEGFADMFDDLAERIVQLGHHPLVTLSEAIKLTRVKEETKTSFHSKDIFKEILEDYKYLEKEFKELSNTAEKEGDKVTVTYADDQLAKLQKSIWMLQAHLA

SEQ ID NO: 6 - protein, 144 aa, Helicobacter pylori
MKTFEILKHLQADAIVLFMKVHNFHWNVKGTDFFNVHKATEEIYEGFADMFDDLAERIVQLGHHPLVTLSEALKLTRVKEETKTSFHSKDIFKEILEDYKYLEKEFKELSNTAEKEGDKVTVTYADDQLAKLQKSIWMLQAHLA

SEQ ID NO: 7 - protein, 144 aa, Helicobacter pylori
MKTFEILKHLQADAIVLFMKVHNFHWNVKGTDFFNVHKATEEIYEGFADMFDDLAERIVQLGHHPLVTLSEAIKLTRVKEETKTSFHSKDIFKEILEDYKHLEKEFKELSNTAEKEGDKVTVTYADDQLAKLQKSIWMLQAHLA

SEQ ID NO: 8 - protein, 144 aa, Helicobacter pylori
MKTFEILKHLQADAIVLFMKVHNFHWNVKGTDFFNVHKATEEIYEGFADMFDDLAERIVQLGHHPLVTLSEALKLTRVKEETKTSFHSKDIFKEILEDYKHLEKEFKELSNTAEKEGDKVTVTYADDQLAKLQKSIWMLQAHLA

SEQ ID NO: 9 - protein, 36 aa, Helicobacter pylori
EILKHLQADAIVLFMKVHNFHWNVKGTDFFNVHKAT

SEQ ID NO: 10 - protein, 34 aa, Helicobacter pylori
NTAEKEGDKVTVTYADDQLAKLQKSIWMLQAHLA

SEQ ID NO: 11 - protein, 36 aa, Helicobacter pylori
ATEEIYEEFADMFDDLAERIVQLGHHPLVTLSEALK

SEQ ID NO: 12 - protein, 36 aa, Helicobacter pylori
LTRVKEETKTSFHSKDIFKEILEDYKHLEKEFKELS

SEQ ID NO: 13 - protein, 20 aa, Homo sapiens
MVLQTQVFISLLLWISGAYG

SEQ ID NO: 14 - protein, 20 aa, Homo sapiens
MYRMQLLSCIALSLALVTNS

SEQ ID NO: 15 - protein, 16 aa, Homo sapiens
MPLLLLLPLLWAGALA

SEQ ID NO: 16 - protein, 21 aa, Artificial Sequence
  Artificial signal peptide for secretion
MWWRLWWLLLLLLLLWPMVWA